European Patent Specification EP 3 778 647 B1, published February 25, 2026. Title: Antibody specifically binding to ErbB3 and use thereof. Applicant: ISU ABXIS. The sequence listing filed with the application follows.

SEQUENCE LISTING (103 sequences)

SEQ ID NO: 1 - protein, 121 aa, Artificial Sequence
  Heavy chain variable region of antibody 442P
EVQLLESGGGLVQPGGSLRLSCAASGFTFSDYDMSWVRQAPGKGLEWVSSIYPDSGSTYYADSVQGRFTISRDNSKNTLYLQMNSLRAEDTAVYYCAKDLHMGPEGPFDYWGQGTLVTVSS

SEQ ID NO: 2 - protein, 121 aa, Artificial Sequence
  Heavy chain variable region of antibody 442S1
EVQLLESGGGLVQPGGSLRLSCAASGFTFSDYDMSWVRQAPGKGLEWVSTIDLDSGSIYYADSVQGRFTISRDNSKNTLYLQMNSLRAEDTAVYYCAKDLHMGPEGPFDYWGQGTLVTVSS

SEQ ID NO: 3 - protein, 121 aa, Artificial Sequence
  Heavy chain variable region of antibody 442S2
EVQLLESGGGLVQPGGSLRLSCAASGFTFSDYDMSWVRQAPGKGLEWVSSIYPDSGSTDYADSVQGRFTISRDNSKNTLYLQMNSLRAEDTAVYYCAKDLHMGPEGPFDYWGQGTLVTVSS

SEQ ID NO: 4 - protein, 121 aa, Artificial Sequence
  Heavy chain variable region of antibody 442S4
EVQLLESGGGLVQPGGSLRLSCAASGFTFSDYDMSWVRQAPGKGLEWVSSIEPDFGSSYYADSVRGRFTISRDNSKNTLYLQMNSLRAEDTAVYYCAKDLHMGPEGPFDYWGQGTLVTVSS

SEQ ID NO: 5 - protein, 121 aa, Artificial Sequence
  Heavy chain variable region of antibody 442S5
EVQLLESGGGLVQPGGSLRLSCAASGFTFSDYDMSWVRQAPGKGLEWVSIIEPDSGSIYYADSVQGRFTISRDNSKNTLYLQMNSLRAEDTAVYYCAKDLHMGPEGPFDYWGQGTLVTVSS

SEQ ID NO: 6 - protein, 121 aa, Artificial Sequence
  Heavy chain variable region of antibody 442S6
EVQLLESGGGLVQPGGSLRLSCAASGFTFSDYDMSWVRQAPGKGLEWVSSIYPDSGSTDYADSVQGRFTISRDNSKNTLYLQMNSLRAEDTAVYYCAKDRHMWPEGPFDYWGQGTLVTVSS

SEQ ID NO: 7 - protein, 121 aa, Artificial Sequence
  Heavy chain variable region of antibody 442S9
EVQLLESGGGLVQPGGSLRLSCAASGFTFSDYDMSWVRQAPGKGLEWVSSIYPDSGSTYYADSVQGRFTISRDNSKNTLYLQMNSLRAEDTAVYYCAKDRHMWPEGPFDYWGQGTLVTVSS

SEQ ID NO: 8 - protein, 121 aa, Artificial Sequence; identical to SEQ ID NO: 7
  Heavy chain variable region of antibody 442S10

SEQ ID NO: 9 - protein, 121 aa, Artificial Sequence; identical to SEQ ID NO: 7
  Heavy chain variable region of antibody 442M3

SEQ ID NO: 10 - protein, 121 aa, Artificial Sequence; identical to SEQ ID NO: 2
  Heavy chain variable region of antibody 442M4

SEQ ID NO: 11 - protein, 121 aa, Artificial Sequence; identical to SEQ ID NO: 2
  Heavy chain variable region of antibody 442M5

SEQ ID NO: 12 - protein, 121 aa, Artificial Sequence
  Heavy chain variable region of antibody 442M6
EVQLLESGGGLVQPGGSLRLSCAASGFTFSDYDMSWVRQAPGKGLEWVSSIEPDSGSTDYADSVQGRFTISRDNSKNTLYLQMNSLRAEDTAVYYCAKDRHMWPEGPFDYWGQGTLVTVSS

SEQ ID NO: 13 - protein, 121 aa, Artificial Sequence
  Heavy chain variable region of antibody 442M7
EVQLLESGGGLVQPGGSLRLSCAASGFTFSDYDMSWVRQAPGKGLEWVSTIEPDSGSTYYADSVQSRFTISRDNSKNTLYLQMNSLRAEDTAVYYCAKDLHMGPEGPFDYWGQGTLVTVSS

SEQ ID NO: 14 - protein, 121 aa, Artificial Sequence; identical to SEQ ID NO: 1
  Heavy chain variable region of antibody 442M8

SEQ ID NO: 15 - protein, 121 aa, Artificial Sequence
  Heavy chain variable region of antibody 442M10
EVQLLESGGGLVQPGGSLRLSCAASGFTFSDYDMSWVRQAPGKGLEWVSSIYPDSGSTDYADSVQGRFTISRDNSKNTLYLQMNSLRAEDTAVYYCAKDLHMWPEGPFDYWGQGTLVTVSS

SEQ ID NO: 16 - protein, 121 aa, Artificial Sequence
  Heavy chain variable region of antibody 442M11
EVQLLESGGGLVQPGGSLRLSCAASGFTFSDYDMSWVRQAPGKGLEWVSTIEPDYGSTLYADSVQGRFTISRDNSKNTLYLQMNSLRAEDTAVYYCAKDLHMGPEGPFDYWGQGTLVTVSS

SEQ ID NO: 17 - protein, 127 aa, Artificial Sequence
  Heavy chain variable region of antibody 472P
EVQLLESGGGLVQPGGSLRLSCAASGFTFSDYDMSWVRQAPGKGLEWVSGISYDGGNTYYADSVKGRFTISRDNSKNTLYLQMNSLRAEDTAVYYCARDPSWCLQDLCYYADGMDVWGQGTLVTVSS

SEQ ID NO: 18 - protein, 127 aa, Artificial Sequence
  Heavy chain variable region of antibody 472S1
EVQLLESGGGLVQPGGSLRLSCAASGFTFSWYDMTWVRQAPGKGLEWVSGISYDGGNTYYADSVKGRFTISRDNSKNTLYLQMNSLRAEDTAVYYCARDPSWCLQDLCYYADGMDVWGQGTLVTVSS

SEQ ID NO: 19 - protein, 127 aa, Artificial Sequence
  Heavy chain variable region of antibody 472S2
EVQLLESGGGLVQPGGSLRLSCAASGFTFSWYDLAWVRQAPGKGLEWVSGISYDGGNTYYADSVKGRFTISRDNSKNTLYLQMNSLRAEDTAVYYCARDPSWCLQDLCYYADGMDVWGQGTLVTVSS

SEQ ID NO: 20 - protein, 127 aa, Artificial Sequence
  Heavy chain variable region of antibody 472S3
EVQLLESGGGLVQPGGSLRLSCAASGFTFSWYDMSWVRQAPGKGLEWVSGISYDGGNTYYADSVKGRFTISRDNSKNTLYLQMNSLRAEDTAVYYCARDPSWCLQDLCYYADGMDVWGQGTLVTVSS

SEQ ID NO: 21 - protein, 127 aa, Artificial Sequence
  Heavy chain variable region of antibody 472S4
EVQLLESGGGLVQPGGSLRLSCAASGFTFSWYDIAWVRQAPGKGLEWVSGISYDGGNTYYADSVKGRFTISRDNSKNTLYLQMNSLRAEDTAVYYCARDPSWCLQDLCYYADGMDVWGQGTLVTVSS

SEQ ID NO: 22 - protein, 127 aa, Artificial Sequence
  Heavy chain variable region of antibody 472M1
EVQLLESGGGLVQPGGSLRLSCAASGFTFSWYDLSWVRQAPGKGLEWVSGISYDGGNTYYADSVKGRFTISRDNSKNTLYLQMNSLRAEDTAVYYCARDPSWCLQDLCYYADGMDVWGQGTLVTVSS

SEQ ID NO: 23 - protein, 121 aa, Artificial Sequence
  Heavy chain variable region of antibody 451P
EVQLLESGGGLVQPGGSLRLSCAASGFTFSDYDMSWVRQAPGKGLEWVSAIYYDSGSIYYADSAKGRFTISRDNSKNTLYLQMNSLRAEDTAVYYCAKDRLFVSDSTFDYWGQGTLVTVSS

SEQ ID NO: 24 - protein, 121 aa, Artificial Sequence
  Heavy chain variable region of antibody 451M1
EVQLLESGGGLVQPGGSLRLSCAASGFTFSDYDMSWVRQAPGKGLEWVSAIYYDSGSIYYADSAKGRFTISRDNSKNTLYLQMNSLRAEDTAVYYCAKDRLFMSDSTFDYWGQGTLVTVSS

SEQ ID NO: 25 - protein, 121 aa, Artificial Sequence
  Heavy chain variable region of antibody 451M2
EVQLLESGGGLVQPGGSLRLSCAASGFTFSDYDMSWVRQAPGKGLEWVSAIYYDSGSIYYADSAKGRFTISRDNSKNTLYLQMNSLRAEDTAVYYCAKDRLFASDSTFDYWGQGTLVTVSS

SEQ ID NO: 26 - protein, 121 aa, Artificial Sequence
  Heavy chain variable region of antibody 451M3
EVQLLESGGGLVQPGGSLRLSCAASGFTFSHYDMSWVRQAPGKGLEWVSAIYYDSGSIYYADSAKGRFTISRDNSKNTLYLQMNSLRAEDTAVYYCAKDRLFASDSTFDYWGQGTLVTVSS

SEQ ID NO: 27 - protein, 121 aa, Artificial Sequence
  Heavy chain variable region of antibody 451M4
EVQLLESGGGLVQPGGSLRLSCAASGFTFSYYDMSWVRQAPGKGLEWVSAIYYDSGSIYYADSAKGRFTISRDNSKNTLYLQMNSLRAEDTAVYYCAKDRLFASDSTFDYWGQGTLVTVSS

SEQ ID NO: 28 - protein, 121 aa, Artificial Sequence
  Heavy chain variable region of antibody 451M5
EVQLLESGGGLVQPGGSLRLSCAASGFTFSDYDMSWVRQAPGKGLEWVSAIYYDSGSIYYADSAKGRFTISRDNSKNTLYLQMNSLRAEDTAVYYCAKDRLFESDSTFDYWGQGTLVTVSS

SEQ ID NO: 29 - protein, 121 aa, Artificial Sequence
  Heavy chain variable region of antibody 451M6
EVQLLESGGGLVQPGGSLRLSCAASGFTFSHYDMSWVRQAPGKGLEWVSAIYYDSGSIYYADSAKGRFTISRDNSKNTLYLQMNSLRAEDTAVYYCAKDRLFESDSTFDYWGQGTLVTVSS

SEQ ID NO: 30 - protein, 121 aa, Artificial Sequence
  Heavy chain variable region of antibody 451M7
EVQLLESGGGLVQPGGSLRLSCAASGFTFSYYDMSWVRQAPGKGLEWVSAIYYDSGSIYYADSAKGRFTISRDNSKNTLYLQMNSLRAEDTAVYYCAKDRLFESDSTFDYWGQGTLVTVSS

SEQ ID NO: 31 - protein, 111 aa, Artificial Sequence
  Light chain variable region of antibody 442P
QSVLTQPPSASGTPGQRVTISCSGSSSNIGSNSVSWYQQLPGTAPKLLIYSDNHRPSGVPDRFSGSKSGTSASLAISGLRSEDEADYYCAAWDSSLSGYVFGGGTKLTVLG

SEQ ID NO: 32 - protein, 111 aa, Artificial Sequence
  Light chain variable region of antibody 442S1
QSVLTQPPSASGTPGQRVTISCSGSSSNIGSNSVSWYQQLPGTAPKLLIYSDNHRPSGVPDRFSGSKSGTSASLAISGLRSEDEADYYCQGWDTSLSGHVFGGGTKLTVLG

SEQ ID NO: 33 - protein, 111 aa, Artificial Sequence; identical to SEQ ID NO: 31
  Light chain variable region of antibody 442S2

SEQ ID NO: 34 - protein, 111 aa, Artificial Sequence; identical to SEQ ID NO: 31
  Light chain variable region of antibody 442S4

SEQ ID NO: 35 - protein, 111 aa, Artificial Sequence; identical to SEQ ID NO: 31
  Light chain variable region of antibody 442S5

SEQ ID NO: 36 - protein, 111 aa, Artificial Sequence
  Light chain variable region of antibody 442S6
QSVLTQPPSASGTPGQRVTISCSGSSSNIGSNSGSWYQQLPGTAPKLLIYADNWRPSGVPDRFSGSKSGTSASLAISGLRSEDEADYYCAAWDSSLSGYVFGGGTKLTVLG

SEQ ID NO: 37 - protein, 111 aa, Artificial Sequence
  Light chain variable region of antibody 442S9
QSVLTQPPSASGTPGQRVTISCSGSSSNIGSNSGSWYQQLPGTAPKLLIYADNHRPSGVPDRFSGSKSGTSASLAISGLRSEDEADYYCAAWDSSLSGYVFGGGTKLTVLG

SEQ ID NO: 38 - protein, 111 aa, Artificial Sequence; identical to SEQ ID NO: 31
  Light chain variable region of antibody 442S10

SEQ ID NO: 39 - protein, 111 aa, Artificial Sequence; identical to SEQ ID NO: 36
  Light chain variable region of antibody 442M3

SEQ ID NO: 40 - protein, 111 aa, Artificial Sequence
  Light chain variable region of antibody 442M4
QSVLTQPPSASGTPGQRVTISCSGSSSNIGSNSVSWYQQLPGTAPKLLIYSDNHRPSGVPDRFSGSKSGTSASLAISGLRSEDEADYYCVGWDSSLYGHVFGGGTKLTVLG

SEQ ID NO: 41 - protein, 111 aa, Artificial Sequence
  Light chain variable region of antibody 442M5
QSVLTQPPSASGTPGQRVTISCSGSSSNIGSNSVSWYQQLPGTAPKLLIYSDNHRPSGVPDRFSGSKSGTSASLAISGLRSEDEADYYCHAWDSSLWGDVFGGGTKLTVLG

SEQ ID NO: 42 - protein, 111 aa, Artificial Sequence; identical to SEQ ID NO: 36
  Light chain variable region of antibody 442M6

SEQ ID NO: 43 - protein, 111 aa, Artificial Sequence; identical to SEQ ID NO: 31
  Light chain variable region of antibody 442M7

SEQ ID NO: 44 - protein, 111 aa, Artificial Sequence
  Light chain variable region of antibody 442M8
QSVLTQPPSASGTPGQRVTISCSGSSSNIGSNSVSWYQQLPGTAPKLLIYSDNHRPSGVPDRFSGSKSGTSASLAISGLRSEDEADYYCHAWDSSLYVDVFGGGTKLTVLG

SEQ ID NO: 45 - protein, 111 aa, Artificial Sequence
  Light chain variable region of antibody 442M10
QSVLTQPPSASGTPGQRVTISCSGSSSNIGSNSVSWYQQLPGTAPKLLIYADNFRPSGVPDRFSGSKSGTSASLAISGLRSEDEADYYCAAWDSSLSGYVFGGGTKLTVLG

SEQ ID NO: 46 - protein, 111 aa, Artificial Sequence
  Light chain variable region of antibody 442M11
QSVLTQPPSASGTPGQRVTISCSGSSSNIGSNSVSWYQQLPGTAPKLLIYSDNHRPSGVPDRFSGSKSGTSASLAISGLRSEDEADYYCHAWDSSLSGDFFGGGTKLTVLG

SEQ ID NO: 47 - protein, 111 aa, Artificial Sequence
  Light chain variable region of antibody 472P
QSVLTQPPSASGTPGQRVTISCSGSSSNIGSNSVSWYQQLPGTAPKLLIYADSNRPSGVPDRFSGSKSGTSASLAISGLRSEDEADYYCGSWDYSLSGYVFGGGTKLTVLG

SEQ ID NO: 48 - protein, 111 aa, Artificial Sequence; identical to SEQ ID NO: 47
  Light chain variable region of antibody 472S1

SEQ ID NO: 49 - protein, 111 aa, Artificial Sequence; identical to SEQ ID NO: 47
  Light chain variable region of antibody 472S2

SEQ ID NO: 50 - protein, 111 aa, Artificial Sequence; identical to SEQ ID NO: 47
  Light chain variable region of antibody 472S3

SEQ ID NO: 51 - protein, 111 aa, Artificial Sequence; identical to SEQ ID NO: 47
  Light chain variable region of antibody 472S4

SEQ ID NO: 52 - protein, 111 aa, Artificial Sequence; identical to SEQ ID NO: 47
  Light chain variable region of antibody 472M1

SEQ ID NO: 53 - protein, 111 aa, Artificial Sequence
  Light chain variable region of antibody 451P
QSVLTQPPSASGTPGQRVTISCSGSPSNIGNNSVTWYQQLPGTAPKLLIYYDSHRPSGVPDRFSGSKSGTSASLAISGLRSEDEADYYCGSWDASLNGYVFGGGTKLTVLG

SEQ ID NO: 54 - protein, 111 aa, Artificial Sequence; identical to SEQ ID NO: 53
  Light chain variable region of antibody 451M1

SEQ ID NO: 55 - protein, 111 aa, Artificial Sequence; identical to SEQ ID NO: 53
  Light chain variable region of antibody 451M2

SEQ ID NO: 56 - protein, 111 aa, Artificial Sequence; identical to SEQ ID NO: 53
  Light chain variable region of antibody 451M3

SEQ ID NO: 57 - protein, 111 aa, Artificial Sequence; identical to SEQ ID NO: 53
  Light chain variable region of antibody 451M4

SEQ ID NO: 58 - protein, 111 aa, Artificial Sequence; identical to SEQ ID NO: 53
  Light chain variable region of antibody 451M5

SEQ ID NO: 59 - protein, 111 aa, Artificial Sequence; identical to SEQ ID NO: 53
  Light chain variable region of antibody 451M6

SEQ ID NO: 60 - protein, 111 aa, Artificial Sequence; identical to SEQ ID NO: 53
  Light chain variable region of antibody 451M7

SEQ ID NO: 61 - protein, 5 aa, Artificial Sequence
  Heavy chain CDR1
DYDMS

SEQ ID NO: 62 - protein, 5 aa, Artificial Sequence
  Heavy chain CDR1
WYDMT

SEQ ID NO: 63 - protein, 5 aa, Artificial Sequence
  Heavy chain CDR1
WYDLA

SEQ ID NO: 64 - protein, 5 aa, Artificial Sequence
  Heavy chain CDR1
WYDMS

SEQ ID NO: 65 - protein, 5 aa, Artificial Sequence
  Heavy chain CDR1
WYDIA

SEQ ID NO: 66 - protein, 5 aa, Artificial Sequence
  Heavy chain CDR1
WYDLS

SEQ ID NO: 67 - protein, 5 aa, Artificial Sequence
  Heavy chain CDR1
HYDMS

SEQ ID NO: 68 - protein, 5 aa, Artificial Sequence
  Heavy chain CDR1
YYDMS

SEQ ID NO: 69 - protein, 17 aa, Artificial Sequence
  Heavy chain CDR2
SIYPDSGSTYYADSVQG

SEQ ID NO: 70 - protein, 17 aa, Artificial Sequence
  Heavy chain CDR2
TIDLDSGSIYYADSVQG

SEQ ID NO: 71 - protein, 17 aa, Artificial Sequence
  Heavy chain CDR2
SIYPDSGSTDYADSVQG

SEQ ID NO: 72 - protein, 17 aa, Artificial Sequence
  Heavy chain CDR2
SIEPDFGSSYYADSVRG

SEQ ID NO: 73 - protein, 17 aa, Artificial Sequence
  Heavy chain CDR2
IIEPDSGSIYYADSVQG

SEQ ID NO: 74 - protein, 17 aa, Artificial Sequence
  Heavy chain CDR2
SIEPDSGSTDYADSVQG

SEQ ID NO: 75 - protein, 17 aa, Artificial Sequence
  Heavy chain CDR2
TIEPDSGSTYYADSVQS

SEQ ID NO: 76 - protein, 17 aa, Artificial Sequence
  Heavy chain CDR2
GISYDGGNTYYADSVKG

SEQ ID NO: 77 - protein, 17 aa, Artificial Sequence
  Heavy chain CDR2
AIYYDSGSIYYADSAKG

SEQ ID NO: 78 - protein, 12 aa, Artificial Sequence
  Heavy chain CDR3
DLHMGPEGPFDY

SEQ ID NO: 79 - protein, 12 aa, Artificial Sequence
  Heavy chain CDR3
DRHMWPEGPFDY

SEQ ID NO: 80 - protein, 12 aa, Artificial Sequence
  Heavy chain CDR3
DLHMWPEGPFDY

SEQ ID NO: 81 - protein, 18 aa, Artificial Sequence
  Heavy chain CDR3
DPSWCLQDLCYYADGMDV

SEQ ID NO: 82 - protein, 12 aa, Artificial Sequence
  Heavy chain CDR3
DRLFVSDSTFDY

SEQ ID NO: 83 - protein, 12 aa, Artificial Sequence
  Heavy chain CDR3
DRLFMSDSTFDY

SEQ ID NO: 84 - protein, 12 aa, Artificial Sequence
  Heavy chain CDR3
DRLFASDSTFDY

SEQ ID NO: 85 - protein, 12 aa, Artificial Sequence
  Heavy chain CDR3
DRLFESDSTFDY

SEQ ID NO: 86 - protein, 13 aa, Artificial Sequence
  Light chain CDR1
SGSSSNIGSNSVS

SEQ ID NO: 87 - protein, 13 aa, Artificial Sequence
  Light chain CDR1
SGSSSNIGSNSGS

SEQ ID NO: 88 - protein, 7 aa, Artificial Sequence
  Light chain CDR2
SDNHRPS

SEQ ID NO: 89 - protein, 7 aa, Artificial Sequence
  Light chain CDR2
ADNWRPS

SEQ ID NO: 90 - protein, 7 aa, Artificial Sequence
  Light chain CDR2
ADNHRPS

SEQ ID NO: 91 - protein, 7 aa, Artificial Sequence
  Light chain CDR2
ADNFRPS

SEQ ID NO: 92 - protein, 7 aa, Artificial Sequence
  Light chain CDR2
ADSNRPS

SEQ ID NO: 93 - protein, 7 aa, Artificial Sequence
  Light chain CDR2
YDSHRPS

SEQ ID NO: 94 - protein, 11 aa, Artificial Sequence
  Light chain CDR3
AAWDSSLSGYV

SEQ ID NO: 95 - protein, 11 aa, Artificial Sequence
  Light chain CDR3
QGWDTSLSGHV

SEQ ID NO: 96 - protein, 11 aa, Artificial Sequence
  Light chain CDR3
VGWDSSLYGHV

SEQ ID NO: 97 - protein, 11 aa, Artificial Sequence
  Light chain CDR3
HAWDSSLWGDV

SEQ ID NO: 98 - protein, 11 aa, Artificial Sequence
  Light chain CDR3
HAWDSSLYVDV

SEQ ID NO: 99 - protein, 11 aa, Artificial Sequence
  Light chain CDR3
HAWDSSLSGDF

SEQ ID NO: 100 - protein, 11 aa, Artificial Sequence
  Light chain CDR3
GSWDYSLSGYV

SEQ ID NO: 101 - protein, 11 aa, Artificial Sequence
  Light chain CDR3
GSWDASLNGYV

SEQ ID NO: 102 - protein, 17 aa, Artificial Sequence
  Heavy chain CDR2
TIEPDYGSTLYADSVQG

SEQ ID NO: 103 - protein, 13 aa, Artificial Sequence
  Light chain CDR1
SGSPSNIGNNSVT